European Patent Application EP 4 782 009 A1, published July 29, 2026. Title: 抗B7H3抗体药物偶联物在制备治疗鼻咽癌和/或肺淋巴上皮瘤样癌的药物中的用途. Applicant: 苏州宜联生物医药有限公司. The sequence listing filed with the application follows.

SEQUENCE LISTING (10 sequences)

SEQ ID NO: 1 - protein, 5 aa, synthetic construct
SYAMN

SEQ ID NO: 2 - protein, 17 aa, synthetic construct
GISGSGGSTYYADSVQG

SEQ ID NO: 3 - protein, 11 aa, synthetic construct
ARSGYDYFFDY

SEQ ID NO: 4 - protein, 12 aa, synthetic construct
RASQRISSSFLA

SEQ ID NO: 5 - protein, 7 aa, synthetic construct
GASSRAT

SEQ ID NO: 6 - protein, 9 aa, synthetic construct
QQYSNSPLT

SEQ ID NO: 7 - protein, 120 aa, synthetic construct
EVQLLESGGGLVQPGGSLRLSCAASGFTFSSYAMNWVRQAPGKGLEWVSGISGSGGSTYYADSVQGRFTISRDNSKNTLYLQMNSLRAEDTAVYYCAKARSGYDYFFDYWGQGTLVTVSS

SEQ ID NO: 8 - protein, 108 aa, synthetic construct
EIVLTQSPGTLSLSPGERATLSCRASQRISSSFLAWYQQKPGQAPSLLIYGASSRATGIPDRFSGSGSGTDFTLTISSLEPEDFAVFYCQQYSNSPLTFGGGTKVEIK

SEQ ID NO: 9 - protein, 450 aa, synthetic construct
EVQLLESGGGLVQPGGSLRLSCAASGFTFSSYAMNWVRQAPGKGLEWVSGISGSGGSTYYADSVQGRFTISRDNSKNTLYLQMNSLRAEDTAVYYCAKARSGYDYFFDYWGQGTLVTVSSASTKGPSVFPLAPSSKSTSGGTAALGCLVKDYFPEPVTVSWNSGALTSGVHTFPAVLQSSGLYSLSSVVTVPSSSLGTQTYICNVNHKPSNTKVDKKVEPKSCDKTHTCPPCPAPELLGGPSVFLFPPKPKDTLMISRTPEVTCVVVDVSHEDPEVKFNWYVDGVEVHNAKTKPREEQYNSTYRVVSVLTVLHQDWLNGKEYKCKVSNKALPAPIEKTISKAKGQPREPQVYTLPPSRDELTKNQVSLTCLVKGFYPSDIAVEWESNGQPENNYKTTPPVLDSDGSFFLYSKLTVDKSRWQQGNVFSCSVMHEALHNHYTQKSLSLSPGK

SEQ ID NO: 10 - protein, 215 aa, synthetic construct
EIVLTQSPGTLSLSPGERATLSCRASQRISSSFLAWYQQKPGQAPSLLIYGASSRATGIPDRFSGSGSGTDFTLTISSLEPEDFAVFYCQQYSNSPLTFGGGTKVEIKRTVAAPSVFIFPPSDEQLKSGTASVVCLLNNFYPREAKVQWKVDNALQSGNSQESVTEQDSKDSTYSLSSTLTLSKADYEKHKVYACEVTHQGLSSPVTKSFNRGEC